European Patent Specification EP 3 768 699 B1, published November 12, 2025. Title: GENETICALLY REPROGRAMMED TREGS EXPRESSING. Applicant: GAVISH-GALILEE BIO APPLICATIONS LTD. GROSS, Gideon WEINSTEIN-MAROM,  Hadas KRONER,  Amit. The sequence listing filed with the application follows.

SEQUENCE LISTING (30 sequences)

SEQ ID NO: 1 - protein, 18 aa, Artificial Sequence
  Synthetic
GSTSGSGKPGSGEGSTKG

SEQ ID NO: 2 - DNA, 39 bp, Artificial Sequence
  Synthetic
ggaggtggcggatccggaggtggctccggaggtggctcc

SEQ ID NO: 3 - protein, 46 aa, Artificial Sequence
  Synthetic
TTTPAPRPPTPAPTIASQPLSLRPEACRPAAGGAVHTRGLDFACDI

SEQ ID NO: 4 - DNA, 138 bp, Artificial Sequence
  Synthetic
accacgacgccagcgccgcgaccaccaacaccggcgcccaccatcgcgtcgcagcccctgtccctgcgcccagaggcgtgccggccagcggcggggggcgcagtgcacacgagggggctggacttcgcctgtgatatc

SEQ ID NO: 5 - protein, 22 aa, Artificial Sequence
  Synthetic
EPKSCDKTHTCPPCPAPELLGG

SEQ ID NO: 6 - DNA, 66 bp, Artificial Sequence
  Artificial sequence
gagcccaaatcttgtgacaaaactcacacatgcccaccgtgcccagcacctgaactcctgggggga

SEQ ID NO: 7 - protein, 64 aa, Artificial Sequence
  Synthetic
RWPESPKAQASSVPTAQPQAEGSLAKATTAPATTRNTGRGGEEKKKEKEKEEQEERETKTPECP

SEQ ID NO: 8 - DNA, 192 bp, Artificial Sequence
  Synthetic
cgctggccagagtctccaaaggcacaggcctcctcagtgcccactgcacaaccccaagcagagggcagcctcgccaaggcaaccacagccccagccaccacccgtaacacaggaagaggaggagaagagaagaagaaggagaaggagaaagaggaacaagaagagagagagacaaagacaccagagtgtccg

SEQ ID NO: 9 - protein, 201 aa, Artificial Sequence
  Synthetic
MVPPPENVRMNSVNFKNILQWESPAFAKGNLTFTAQYLSYRIFQDKCMNTTLTECDFSSLSKYGDHTLRVRAEFADEHSDWVNITFCPVDDTIIGPPGMQVEVLADSLHMRFLAPKIENEYETWTMKNVYNSWTYNVQYWKNGTDEKFQITPQYDFEVLRNLEPWTTYCVQVRGFLPDRNKAGEWSEPVCEQTTHDETVPS

SEQ ID NO: 10 - DNA, 603 bp, Artificial Sequence
  Synthetic
atggtaccacctcccgaaaatgtcagaatgaattctgttaatttcaagaacattctacagtgggagtcacctgcttttgccaaagggaacctgactttcacagctcagtacctaagttataggatattccaagataaatgcatgaatactaccttgacggaatgtgatttctcaagtctttccaagtatggtgaccacaccttgagagtcagggctgaatttgcagatgagcattcagactgggtaaacatcaccttctgtcctgtggatgacaccattattggaccccctggaatgcaagtagaagtacttgctgattctttacatatgcgtttcttagcccctaaaattgagaatgaatacgaaacttggactatgaagaatgtgtataactcatggacttataatgtgcaatactggaaaaacggtactgatgaaaagtttcaaattactccccagtatgactttgaggtcctcagaaacctggagccatggacaacttattgtgttcaagttcgagggtttcttcctgatcggaacaaagctggggaatggagtgagcctgtctgtgagcaaacaacccatgacgaaacggtcccctcc

SEQ ID NO: 11 - protein, 9 aa, Artificial Sequence
  Synthetic
GGGGSGGGS

SEQ ID NO: 12 - DNA, 27 bp, Artificial Sequence
  Synthetic
ggaggtggcggatccggaggtggctcc

SEQ ID NO: 13 - protein, 13 aa, Artificial Sequence
  Synthetic
GGGGSGGGSGGGS

SEQ ID NO: 14 - DNA, 39 bp, Artificial Sequence; identical to SEQ ID NO: 2
  Synthetic

SEQ ID NO: 15 - protein, 28 aa, Artificial Sequence
  Synthetic
GGGGSGGGSGGGSSSGGGGSGGGSGGGS

SEQ ID NO: 16 - DNA, 84 bp, Artificial Sequence
  Synthetic
ggaggtggcggatccggaggtggctccggaggtggctcctcgagcggaggtggcggatccggaggtggctccggaggtggctcc

SEQ ID NO: 17 - protein, 8 aa, Artificial Sequence
  Synthetic
SSQPTIPI

SEQ ID NO: 18 - DNA, 24 bp, Artificial Sequence
  Synthetic
tcgagccagcccaccatccccatc

SEQ ID NO: 19 - protein, 57 aa, Artificial Sequence
  Synthetic
VGIIAGLVLFGAVITGAVVAAVMWRRKSSDRKGGSYSQAASSDSAQGSDVSLTACKV

SEQ ID NO: 20 - DNA, 174 bp, Artificial Sequence
  Synthetic
gtgggcatcattgctggcctggttctctttggagctgtgatcactggagctgtggtcgctgctgtgatgtggaggaggaagagctcagatagaaaaggagggagctactctcaggctgcaagcagtgacagtgcccagggctctgatgtgtctctcacagcttgtaaagtgtga

SEQ ID NO: 21 - protein, 27 aa, Artificial Sequence
  Synthetic
FWVLVVVGGVLACYSLLVTVAFIIFWV

SEQ ID NO: 22 - DNA, 81 bp, Artificial Sequence
  Synthetic
ttctgggtgttggtcgttgtgggtggtgtcctggcgtgttattcactgttggttactgtggcttttataattttctgggtg

SEQ ID NO: 23 - protein, 105 aa, Artificial Sequence
  Synthetic
WMVAVILMASVFMVCLALLGCFALLWCVYKKTKYAFSPRNSLPQHLKEFLGHPHHNTLLFFSFPLSDENDVFDKLSVIAEDSESGKQNPGDSCSLGTPPGQGPQS

SEQ ID NO: 24 - DNA, 318 bp, Artificial Sequence
  Synthetic
tggatggtggccgtcatcctcatggcctcggtcttcatggtctgcctggcactcctcggctgcttcgccttgctgtggtgcgtttacaagaagacaaagtacgccttctcccctaggaattctcttccacagcacctgaaagagtttttgggccatcctcatcataacacacttctgtttttctcctttccattgtcggatgagaatgatgtttttgacaagctaagtgtcattgcagaagactctgagagcggcaagcagaatcctggtgacagctgcagcctcgggaccccgcctgggcaggggccccaaagctag

SEQ ID NO: 25 - protein, 434 aa, Artificial Sequence
  Synthetic
MHSSALLCCLVLLTGVRASPGQGTQSENSCTHFPGNLPNMLRDLRDAFSRVKTFFQMKDQLDNLLLKESLLEDFKGYLGCQALSEMIQFYLEEVMPQAENQDPDIKAHVNSLGENLKTLRLRLRRCHRFLPCENKSKAVEQVKNAFNKLQEKGIYKAMSEFDIFINYIEAYMTMKIRNGSTSGSGKPGSGEGSTKGSPGQGTQSENSCTHFPGNLPNMLRDLRDAFSRVKTFFQMKDQLDNLLLKESLLEDFKGYLGCQALSEMIQFYLEEVMPQAENQDPDIKAHVNSLGENLKTLRLRLRRCHRFLPCENKSKAVEQVKNAFNKLQEKGIYKAMSEFDIFINYIEAYMTMKIRNGGGGSGGGSGGGSSSQPTIPIVGIIAGLVLFGAVITGAVVAAVMWRRKSSDRKGGSYSQAASSDSAQGSDVSLTACKV

SEQ ID NO: 26 - DNA, 1305 bp, Artificial Sequence
  Synthetic
atgcacagctcagcactgctctgttgcctggtcctcctgactggggtgagggccagcccaggccagggcacccagtctgagaacagctgcacccacttcccaggcaacctgcctaacatgcttcgagatctccgagatgccttcagcagagtgaagactttctttcaaatgaaggatcagctggacaacttgttgttaaaggagtccttgctggaggactttaagggttacctgggttgccaagccttgtctgagatgatccagttttacctggaggaggtgatgccccaagctgagaaccaagacccagacatcaaggcgcatgtgaactccctgggggagaacctgaagaccctcaggctgaggctacggcgctgtcatcgatttcttccctgtgaaaacaagagcaaggccgtggagcaggtgaagaatgcctttaataagctccaagagaaaggcatctacaaagccatgagtgagtttgacatcttcatcaactacatagaagcctacatgacaatgaagatacgaaacggcagtacttcgggcagtggtaagcccgggagtggtgagggtagtactaagggtagcccaggccagggcacccagtctgagaacagctgcacccacttcccaggcaacctgcctaacatgcttcgagatctccgagatgccttcagcagagtgaagactttctttcaaatgaaggatcagctggacaacttgttgttaaaggagtccttgctggaggactttaagggttacctgggttgccaagccttgtctgagatgatccagttttacctggaggaggtgatgccccaagctgagaaccaagacccagacatcaaggcgcatgtgaactccctgggggagaacctgaagaccctcaggctgaggctacggcgctgtcatcgatttcttccctgtgaaaacaagagcaaggccgtggagcaggtgaagaatgcctttaataagctccaagagaaaggcatctacaaagccatgagtgagtttgacatcttcatcaactacatagaagcctacatgacaatgaagatacgaaacggaggtggcggatccggaggtggctccggaggtggctcctcgagccagcccaccatccccatcgtgggcatcattgctggcctggttctctttggagctgtgatcactggagctgtggtcgctgctgtgatgtggaggaggaagagctcagatagaaaaggagggagctactctcaggctgcaagcagtgacagtgcccagggctctgatgtgtctctcacagcttgtaaagtgtga

SEQ ID NO: 27 - protein, 448 aa, Artificial Sequence
  Synthetic
MHSSALLCCLVLLTGVRASPGQGTQSENSCTHFPGNLPNMLRDLRDAFSRVKTFFQMKDQLDNLLLKESLLEDFKGYLGCQALSEMIQFYLEEVMPQAENQDPDIKAHVNSLGENLKTLRLRLRRCHRFLPCENKSKAVEQVKNAFNKLQEKGIYKAMSEFDIFINYIEAYMTMKIRNGSTSGSGKPGSGEGSTKGSPGQGTQSENSCTHFPGNLPNMLRDLRDAFSRVKTFFQMKDQLDNLLLKESLLEDFKGYLGCQALSEMIQFYLEEVMPQAENQDPDIKAHVNSLGENLKTLRLRLRRCHRFLPCENKSKAVEQVKNAFNKLQEKGIYKAMSEFDIFINYIEAYMTMKIRNGGGGSGGGSGGGSSSGGGGSGGGSGGGSSSQPTIPIVGIIAGLVLFGAVITGAVVAAVMWRRKSSDRKGGSYSQAASSDSAQGSDVSLTACK

SEQ ID NO: 28 - DNA, 1350 bp, Artificial Sequence
  Synthetic
atgcacagctcagcactgctctgttgcctggtcctcctgactggggtgagggccagcccaggccagggcacccagtctgagaacagctgcacccacttcccaggcaacctgcctaacatgcttcgagatctccgagatgccttcagcagagtgaagactttctttcaaatgaaggatcagctggacaacttgttgttaaaggagtccttgctggaggactttaagggttacctgggttgccaagccttgtctgagatgatccagttttacctggaggaggtgatgccccaagctgagaaccaagacccagacatcaaggcgcatgtgaactccctgggggagaacctgaagaccctcaggctgaggctacggcgctgtcatcgatttcttccctgtgaaaacaagagcaaggccgtggagcaggtgaagaatgcctttaataagctccaagagaaaggcatctacaaagccatgagtgagtttgacatcttcatcaactacatagaagcctacatgacaatgaagatacgaaacggcagtacttcgggcagtggtaagcccgggagtggtgagggtagtactaagggtagcccaggccagggcacccagtctgagaacagctgcacccacttcccaggcaacctgcctaacatgcttcgagatctccgagatgccttcagcagagtgaagactttctttcaaatgaaggatcagctggacaacttgttgttaaaggagtccttgctggaggactttaagggttacctgggttgccaagccttgtctgagatgatccagttttacctggaggaggtgatgccccaagctgagaaccaagacccagacatcaaggcgcatgtgaactccctgggggagaacctgaagaccctcaggctgaggctacggcgctgtcatcgatttcttccctgtgaaaacaagagcaaggccgtggagcaggtgaagaatgcctttaataagctccaagagaaaggcatctacaaagccatgagtgagtttgacatcttcatcaactacatagaagcctacatgacaatgaagatacgaaacggaggtggcggatccggaggtggctccggaggtggctcctcgagcggaggtggcggatccggaggtggctccggaggtggctcctcgagccagcccaccatccccatcgtgggcatcattgctggcctggttctctttggagctgtgatcactggagctgtggtcgctgctgtgatgtggaggaggaagagctcagatagaaaaggagggagctactctcaggctgcaagcagtgacagtgcccagggctctgatgtgtctctcacagcttgtaaagtgtga

SEQ ID NO: 29 - protein, 677 aa, Artificial Sequence
  Synthetic
MHSSALLCCLVLLTGVRASPGQGTQSENSCTHFPGNLPNMLRDLRDAFSRVKTFFQMKDQLDNLLLKESLLEDFKGYLGCQALSEMIQFYLEEVMPQAENQDPDIKAHVNSLGENLKTLRLRLRRCHRFLPCENKSKAVEQVKNAFNKLQEKGIYKAMSEFDIFINYIEAYMTMKIRNGSTSGSGKPGSGEGSTKGSPGQGTQSENSCTHFPGNLPNMLRDLRDAFSRVKTFFQMKDQLDNLLLKESLLEDFKGYLGCQALSEMIQFYLEEVMPQAENQDPDIKAHVNSLGENLKTLRLRLRRCHRFLPCENKSKAVEQVKNAFNKLQEKGIYKAMSEFDIFINYIEAYMTMKIRNGGGGSGGGSGGGSSSMVPPPENVRMNSVNFKNILQWESPAFAKGNLTFTAQYLSYRIFQDKCMNTTLTECDFSSLSKYGDHTLRVRAEFADEHSDWVNITFCPVDDTIIGPPGMQVEVLADSLHMRFLAPKIENEYETWTMKNVYNSWTYNVQYWKNGTDEKFQITPQYDFEVLRNLEPWTTYCVQVRGFLPDRNKAGEWSEPVCEQTTHDETVPSWMVAVILMASVFMVCLALLGCFALLWCVYKKTKYAFSPRNSLPQHLKEFLGHPHHNTLLFFSFPLSDENDVFDKLSVIAEDSESGKQNPGDSCSLGTPPGQGPQS

SEQ ID NO: 30 - DNA, 2034 bp, Artificial Sequence
  Synthetic
atgcacagctcagcactgctctgttgcctggtcctcctgactggggtgagggccagcccaggccagggcacccagtctgagaacagctgcacccacttcccaggcaacctgcctaacatgcttcgagatctccgagatgccttcagcagagtgaagactttctttcaaatgaaggatcagctggacaacttgttgttaaaggagtccttgctggaggactttaagggttacctgggttgccaagccttgtctgagatgatccagttttacctggaggaggtgatgccccaagctgagaaccaagacccagacatcaaggcgcatgtgaactccctgggggagaacctgaagaccctcaggctgaggctacggcgctgtcatcgatttcttccctgtgaaaacaagagcaaggccgtggagcaggtgaagaatgcctttaataagctccaagagaaaggcatctacaaagccatgagtgagtttgacatcttcatcaactacatagaagcctacatgacaatgaagatacgaaacggcagtacttcgggcagtggtaagcccgggagtggtgagggtagtactaagggtagcccaggccagggcacccagtctgagaacagctgcacccacttcccaggcaacctgcctaacatgcttcgagatctccgagatgccttcagcagagtgaagactttctttcaaatgaaggatcagctggacaacttgttgttaaaggagtccttgctggaggactttaagggttacctgggttgccaagccttgtctgagatgatccagttttacctggaggaggtgatgccccaagctgagaaccaagacccagacatcaaggcgcatgtgaactccctgggggagaacctgaagaccctcaggctgaggctacggcgctgtcatcgatttcttccctgtgaaaacaagagcaaggccgtggagcaggtgaagaatgcctttaataagctccaagagaaaggcatctacaaagccatgagtgagtttgacatcttcatcaactacatagaagcctacatgacaatgaagatacgaaacggaggtggcggatccggaggtggctccggaggtggctcctcgagcatggtaccacctcccgaaaatgtcagaatgaattctgttaatttcaagaacattctacagtgggagtcacctgcttttgccaaagggaacctgactttcacagctcagtacctaagttataggatattccaagataaatgcatgaatactaccttgacggaatgtgatttctcaagtctttccaagtatggtgaccacaccttgagagtcagggctgaatttgcagatgagcattcagactgggtaaacatcaccttctgtcctgtggatgacaccattattggaccccctggaatgcaagtagaagtacttgctgattctttacatatgcgtttcttagcccctaaaattgagaatgaatacgaaacttggactatgaagaatgtgtataactcatggacttataatgtgcaatactggaaaaacggtactgatgaaaagtttcaaattactccccagtatgactttgaggtcctcagaaacctggagccatggacaacttattgtgttcaagttcgagggtttcttcctgatcggaacaaagctggggaatggagtgagcctgtctgtgagcaaacaacccatgacgaaacggtcccctcctggatggtggccgtcatcctcatggcctcggtcttcatggtctgcctggcactcctcggctgcttcgccttgctgtggtgcgtttacaagaagacaaagtacgccttctcccctaggaattctcttccacagcacctgaaagagtttttgggccatcctcatcataacacacttctgtttttctcctttccattgtcggatgagaatgatgtttttgacaagctaagtgtcattgcagaagactctgagagcggcaagcagaatcctggtgacagctgcagcctcgggaccccgcctgggcaggggccccaaagctag